European Patent Application EP 4 218 788 A1, published August 2, 2023. Title: NOVEL USE OF PEPTIDE FOR INHIBITING FUNCTIONS AND EXPRESSIONS OF MULTIPLE DISEASE BIOMARKERS. Applicant: NIBEC CO., LTD. Application KR PCT/KR2019/011037, filed August 29, 2019. The sequence listing filed with the application follows.

SEQUENCE LISTING (8 sequences)

SEQ ID NO: 1 - protein, 15 aa, synthetic construct
GKCSTRGRKCCRRKK

SEQ ID NO: 2 - protein, 15 aa, synthetic construct
GKCSTRGRKCMRRKK

SEQ ID NO: 3 - protein, 15 aa, synthetic construct
GKCSTRGRKMCRRKK

SEQ ID NO: 4 - protein, 15 aa, synthetic construct
GKCSTRGRKMMRRKK

SEQ ID NO: 5 - protein, 15 aa, synthetic construct
GKMSTRGRKCCRRKK

SEQ ID NO: 6 - protein, 15 aa, synthetic construct
GKMSTRGRKMCRRKK

SEQ ID NO: 7 - protein, 15 aa, synthetic construct
GKMSTRGRKCMRRKK

SEQ ID NO: 8 - protein, 15 aa, synthetic construct
GKMSTRGRKMMRRKK